European Patent Application EP 4 748 852 A1, published May 27, 2026. Title: 一种角蛋白CF7、制法和其药物组合物与用途. Applicant: 中国医学科学院药物研究所. The sequence listing filed with the application follows.

SEQUENCE LISTING (2 sequences)

SEQ ID NO: 1 - protein, 404 aa, unidentified
MSYNCSLPNLSCRSSFSARPCVPPSCRSCTLPGACNIPANVGSCSWFCEGSFNGSEKETMQFLNDRLASYLEKVRQLERDNAELESLIRERSQQQEPEVCPNYQSYFRTIEELQQKILCTKSENARLVVQIDNAKLAADDFRTKYETELGLRQLVESDINGLRRILDELTLCKADLEAQVESLKEELLCLKQNHEQEVNTLRSQLGDRLNVEVDAAPTVDLNRVLNETRSQYEALVETNRRDVEEWFTTQTEELNRQVVSSSEQLQSYQAEIIELRRTVNALEVELQAQHNLRDSLENTLMETEARYSAQLSQVQGLITSVESQLAEIRSDLERQNQEYQVLLDVRARLESEINTYRGLLESEDCKLPCNPCATTNACDKSIGSCISNPCAPRTRYGPCNTFVR

SEQ ID NO: 2 - DNA, 1212 bp, unidentified
  source 1..1212: mol_type = other DNA
atgagctataactgcagcctgccgaacctgagctgccgctcaagctttagcgcgcgtccttgtgttcctccgagctgtcgtagctgtaccttaccgggcgcgtgtaacattcctgcgaacgttggcagctgcagctggttttgcgaaggcagctttaacggcagcgaaaaagaaaccatgcagtttctgaacgatcgcctggcgagctatctggaaaaagtgcgccagctggaacgcgataacgcggaattagaaagcctgattcgcgaacgcagccagcagcaggaaccggaagtttgccctaattatcagagctattttcgcaccattgaggaactgcagcagaaaattctgtgcaccaaaagcgaaaacgcgcgcctggtggtgcagattgataacgcgaaactggcggcggatgattttcgcaccaaatatgaaaccgaactgggcctgcgccagctggtggaaagcgatattaacggcctgcgccgcattctggatgaactgaccttatgcaaagcggatctggaagcgcaggtggaaagcctgaaagaagaactgctgtgcctgaaacagaaccatgaacaggaagtgaacaccctgcgcagccagctgggtgatcgtctgaacgttgaagttgatgcggcgccgaccgtggatttaaaccgcgttttgaacgaaacccgcagccagtatgaagcgctggtggaaaccaaccgccgcgatgttgaagaatggtttaccacccagaccgaagaactgaaccgccaggtggtgagcagcagcgaacaattacagagctatcaggcggaaattattgagctgcgccgcaccgtgaacgcgctggaagttgaattacaggcgcagcataacctgcgcgatagcctggaaaacaccctgatggaaaccgaagcgcgctatagcgcgcagctgagccaagttcaaggcttaattaccagcgttgaaagccagctggcggaaattcgcagcgatctggaacgccagaaccaggaatatcaggtgctgctggatgtgcgcgcgcgcttagaaagcgaaattaacacctatcgcggcctgctggaaagcgaagattgcaaactgccgtgcaacccgtgcgcgaccactaatgcgtgtgataaaagcattggcagctgcattagcaacccgtgcgcgccgcgtactcgttatggtccttgtaatacctttgtgcgc